European Patent Application EP 4 279 596 A1, published November 22, 2023. Title: Chimeric target factor receptor. Applicant: NATIONAL UNIVERSITY CORPORATION TOKAI NATIONAL HIGHER EDUCATION AND RESEARCH SYSTEM. The sequence listing filed with the application follows.

SEQUENCE LISTING (20 sequences)

SEQ ID NO: 1 - protein, 268 aa, Artificial Sequence
  Her2 scFv
DFQVQIFSFLLISASVIMSRGDIQMTQSPSSLSASVGDRVTITCRASQDVNTAVAWYQQKPGKAPKLLIYSASFLYSGVPSRFSGSRSGTDFTLTISSLQPEDFATYYCQQHYTTPPTFGQGTKVEIKRTGSTSGSGKPGSGEGSEVQLVESGGGLVQPGGSLRLSCAASGFNIKDTYIHWVRQAPGKGLEWVARIYPTNGYTRYADSVKGRFTISADTSKNTAYLQMNSLRAEDTAVYYCSRWGGDGFYAMDVWGQGTLVTVSSAAA

SEQ ID NO: 2 - protein, 109 aa, Artificial Sequence
  CD28
IEVMYPPPYLDNEKSNGTIIHVKGKHLCPSPLFPGPSKPFWVLVVVGGVLACYSLLVTVAFIIFWVRSKRSRLLHSDYMNMTPRRPGPTRKHYQPYAPPRDFAAYRSKL

SEQ ID NO: 3 - protein, 185 aa, Artificial Sequence
  TLR1
SYLDLPWYLRMVCQWTQTRRRARNIPLEELQRNLQFHAFISYSGHDSFWVKNELLPNLEKEGMQICLHERNFVPGKSIVENIITCIEKSYKSIFVLSPNFVQSEWCHYELYFAHHNLFHEGSNSLILILLEPIPQYSIPSSYHKLKSLMARRTYLEWPKEKSKRGLFWANLRAAINIKLTEQAKK

SEQ ID NO: 4 - protein, 174 aa, Artificial Sequence
  TLR2
RFHGLWYMKMMWAWLQAKRKPRKAPSRNICYDAFVSYSERDAYWVENLMVQELENFNPPFKLCLHKRDFIPGKWIIDNIIDSIEKSHKTVFVLSENFVKSEWCKYELDFSHFRLFDENNDAAILILLEPIEKKAIPQRFCKLRKIMNTKTYLEWPMDEAQREGFWVNLRAAIKS

SEQ ID NO: 5 - protein, 178 aa, Artificial Sequence
  TLR3
GWRISFYWNVSVHRVLGFKEIDRQTEQFEYAAYIIHAYKDKDWVWEHFSSMEKEDQSLKFCLEERDFEAGVFELEAIVNSIKRSRKIIFVITHHLLKDPLCKRFKVHHAVQQAIEQNLDSIILVFLEEIPDYKLNHALCLRRGMFKSHCILNWPVQKERIGAFRHKLQVALGSKNSVH

SEQ ID NO: 6 - protein, 186 aa, Artificial Sequence
  TLR4
FYFHLMLLAGCIKYGRGENIYDAFVIYSSQDEDWVRNELVKNLEEGVPPFQLCLHYRDFIPGVAIAANIIHEGFHKSRKVIVVVSQHFIQSRWCIFEYEIAQTWQFLSSRAGIIFIVLQKVEKTLLRQQVELYRLLSRNTYLEWEDSVLGRHIFWRRLRKALLDGKSWNPEGTVGTGCNWQEATSI

SEQ ID NO: 7 - protein, 192 aa, Artificial Sequence
  TLR9
WDLWYCFHLCLAWLPWRGRQSGRDEDALPYDAFVVFDKTQSAVADWVYNELRGQLEECRGRWALRLCLEERDWLPGKTLFENLWASVYGSRKTLFVLAHTDRVSGLLRASFLLAQQRLLEDRKDVVVLVILSPDGRRSRYVRLRQRLCRQSVLLWPHQPSGQRSFWAQLGMALTRDNHHFYNRNFCQGPTAE

SEQ ID NO: 8 - protein, 62 aa, Artificial Sequence
  CD40
KKVAKKPTNKAPHPKQEPQEINFPDDLPGSNTAAPVQETLHGCQPVTQEDGKESRISVQERQ

SEQ ID NO: 9 - DNA, 804 bp, Artificial Sequence
  Her2 scFV
gattttcaggtgcagattttcagcttcctgctaatcagtgcctcagtcataatgtccagaggagatatccagatgacccagtccccgagctccctgtccgcctctgtgggcgatagggtcaccatcacctgccgtgccagtcaggatgtgaatactgctgtagcctggtatcaacagaaaccaggaaaagctccgaaactactgatttactcggcatccttcctttattctggagtcccttctcgcttctctggatctagatctgggacggatttcactctgaccatcagcagtctgcagccggaagacttcgcaacttattactgtcagcaacattatactactcctcccacgttcggacagggtaccaaggtggagatcaaacgcactgggtctacatctggatctgggaagccgggttctggtgagggttctgaggttcagctggtggagtctggcggtggcctggtgcagccagggggctcactccgtttgtcctgtgcagcttctggcttcaacattaaagacacctatatacactgggtgcgtcaggccccgggtaagggcctggaatgggttgcaaggatttatcctacgaatggttatactagatatgccgatagcgtcaagggccgtttcactataagcgcagacacatccaaaaacacagcctacctgcagatgaacagcctgcgtgctgaggacactgccgtctattattgttctagatggggaggggacggcttctatgctatggacgtgtggggtcaaggaaccctggtcaccgtctcctcggcggccgca

SEQ ID NO: 10 - DNA, 327 bp, Artificial Sequence
  CD28
attgaagttatgtatcctcctccttacctagacaatgagaagagcaatggaaccattatccatgtgaaagggaaacacctttgtccaagtcccctatttcccggaccttctaagcccttttgggtgctggtggtggttgggggagtcctggcttgctatagcttgctagtaacagtggcctttattattttctgggtgaggagtaagaggagcaggctcctgcacagtgactacatgaacatgactccccgccgccccgggcccacccgcaagcattaccagccctatgccccaccacgcgacttcgcagcctatcgctccaagctt

SEQ ID NO: 11 - DNA, 555 bp, Artificial Sequence
  TLR1
agctacttggatctgccctggtatctcaggatggtgtgccagtggacccagacccggcgcagggccaggaacatacccttagaagaactccaaagaaatctccagtttcatgcatttatttcatatagtgggcacgattctttctgggtgaagaatgaattattgccaaacctagagaaagaaggtatgcagatttgccttcatgagagaaactttgttcctggcaagagcattgtggaaaatatcatcacctgcattgagaagagttacaagtccatctttgttttgtctcccaactttgtccagagtgaatggtgccattatgaactctactttgcccatcacaatctctttcatgaaggatctaatagcttaatcctgatcttgctggaacccattccgcagtactccattcctagcagttatcacaagctcaaaagtctcatggccaggaggacttatttggaatggcccaaggaaaagagcaaacgtggccttttttgggctaacttaagggcagccattaatattaagctgacagagcaagcaaagaaa

SEQ ID NO: 12 - DNA, 522 bp, Artificial Sequence
  TLR2
cgtttccatggcctgtggtatatgaaaatgatgtgggcctggctccaggccaaaaggaagcccaggaaagctcccagcaggaacatctgctatgatgcatttgtttcttacagtgagcgggatgcctactgggtggagaaccttatggtccaggagctggagaacttcaatccccccttcaagttgtgtcttcataagcgggacttcattcctggcaagtggatcattgacaatatcattgactccattgaaaagagccacaaaactgtctttgtgctttctgaaaactttgtgaagagtgagtggtgcaagtatgaactggacttctcccatttccgtctttttgatgagaacaatgatgctgccattctcattcttctggagcccattgagaaaaaagccattccccagcgcttctgcaagctgcggaagataatgaacaccaagacctacctggagtggcccatggacgaggctcagcgggaaggattttgggtaaatctgagagctgcgataaagtcc

SEQ ID NO: 13 - DNA, 534 bp, Artificial Sequence
  TLR3
ggctggaggatatctttttattggaatgtttcagtacatcgagttcttggtttcaaagaaatagacagacagacagaacagtttgaatatgcagcatatataattcatgcctataaagataaggattgggtctgggaacatttctcttcaatggaaaaggaagaccaatctctcaaattttgtctggaagaaagggactttgaggcgggtgtttttgaactagaagcaattgttaacagcatcaaaagaagcagaaaaattatttttgttataacacaccatctattaaaagacccattatgcaaaagattcaaggtacatcatgcagttcaacaagctattgaacaaaatctggattccattatattggttttccttgaggagattccagattataaactgaaccatgcactctgtttgcgaagaggaatgtttaaatctcactgcatcttgaactggccagttcagaaagaacggataggtgcctttcgtcataaattgcaagtagcacttggatccaaaaactctgtacat

SEQ ID NO: 14 - DNA, 558 bp, Artificial Sequence
  TLR4
ttctattttcacctgatgcttcttgctggctgcataaagtatggtagaggtgaaaacatctatgatgcctttgttatctactcaagccaggatgaggactgggtaaggaatgagctagtaaagaatttagaagaaggggtgcctccatttcagctctgccttcactacagagactttattcccggtgtggccattgctgccaacatcatccatgaaggtttccataaaagccgaaaggtgattgttgtggtgtcccagcacttcatccagagccgctggtgtatctttgaatatgagattgctcagacctggcagtttctgagcagtcgtgctggtatcatcttcattgtcctgcagaaggtggagaagaccctgctcaggcagcaggtggagctgtaccgccttctcagcaggaacacttacctggagtgggaggacagtgtcctggggcggcacatcttctggagacgactcagaaaagccctgctggatggtaaatcatggaatccagaaggaacagtgggtacaggatgcaattggcaggaagcaacatctatc

SEQ ID NO: 15 - DNA, 576 bp, Artificial Sequence
  TLR9
tgggacctctggtactgcttccacctgtgcctggcctggcttccctggcgggggcggcaaagtgggcgagatgaggatgccctgccctacgatgccttcgtggtcttcgacaaaacgcagagcgcagtggcagactgggtgtacaacgagcttcgggggcagctggaggagtgccgtgggcgctgggcactccgcctgtgcctggaggaacgcgactggctgcctggcaaaaccctctttgagaacctgtgggcctcggtctatggcagccgcaagacgctgtttgtgctggcccacacggaccgggtcagtggtctcttgcgcgccagcttcctgctggcccagcagcgcctgctggaggaccgcaaggacgtcgtggtgctggtgatcctgagccctgacggccgccgctcccgctacgtgcggctgcgccagcgcctctgccgccagagtgtcctcctctggccccaccagcccagtggtcagcgcagcttctgggcccagctgggcatggccctgaccagggacaaccaccacttctataaccggaacttctgccagggacccacggccgaa

SEQ ID NO: 16 - DNA, 186 bp, Artificial Sequence
  CD40
aaaaaggtggccaagaagccaaccaataaggccccccaccccaagcaggaaccccaggagatcaattttcccgacgatcttcctggctccaacactgctgctccagtgcaggagactttacatggatgccaaccggtcacccaggaggatggcaaagagagtcgcatctcagtgcaggagagacag

SEQ ID NO: 17 - protein, 243 aa, Artificial Sequence
  MSLN scFV
QVQLQQSGPELEKPGASVKISCKASGYSFTGYTMNWVKQSHGKSLEWIGLITPYNGASSYNQKFRGKATLTVDKSSSTAYMDLLSLTSEDSAVYFCARGGYDGRGFDYWGQGTTVTVSSGVGGSGGGGSGGGGSDIELTQSPAIMSASPGEKVTMTCSASSSVSYMHWYQQKSGTSPKRWIYDTSKLASGVPGRFSGSGSGNSYSLTISSVEAEDDATYYCQQWSGYPLTFGAGTKLEIKAAA

SEQ ID NO: 18 - DNA, 729 bp, Artificial Sequence
  MSLN scFV
caggtacaactgcagcagtctgggcctgagctggagaagcctggcgcttcagtgaagatatcctgcaaggcttctggttactcattcactggctacaccatgaactgggtgaagcagagccatggaaagagccttgagtggattggacttattactccttacaatggtgcttctagctacaaccagaagttcaggggcaaggccacattaactgtagacaagtcatccagcacagcctacatggacctcctcagtctgacatctgaagactctgcagtctatttctgtgcaagggggggttacgacgggaggggttttgactactggggccaagggaccacggtcaccgtctcctcaggtgtaggcggttcaggcggcggtggctctggcggtggcggatcggacatcgagctcactcagtctccagcaatcatgtctgcatctccaggggagaaggtcaccatgacctgcagtgccagctcaagtgtaagttacatgcactggtaccagcagaagtcaggcacctcccccaaaagatggatttatgacacatccaaactggcttctggagtcccaggtcgcttcagtggcagtgggtctggaaactcttactctctcacaatcagcagcgtggaggctgaagatgatgcaacttattactgccagcagtggagtggttaccctctcacgttcggtgctgggacaaagttggaaataaaagcggccgct

SEQ ID NO: 19 - protein, 22 aa, Artificial Sequence
  GMCSFR
MLLLVTSLLLCELPHPAFLLIP

SEQ ID NO: 20 - DNA, 66 bp, Artificial Sequence
  GMCSFR
atgcttctcctggtgacaagccttctgctctgtgagttaccacacccagcattcctcctgatccca